European Patent Specification EP 3 427 575 B1, published June 10, 2026. Title: ENDIVE PLANT THAT SHOWS REDUCED BROWNING. Applicant: Rijk Zwaan Zaadteelt en Zaadhandel B.V. The sequence listing filed with the application follows.

SEQUENCE LISTING (4 sequences)

SEQ ID NO: 1 - DNA, 2136 bp, Cichorium endivia
atggagaacggtaatcatgttaatggagtcgttaaggagttttgcatcaaggatccgttgaactggggggttgcggcggaggcgttgaccgggagtcaccttgatgaggtgaagaagatggtgaaggagttcaggaagccggtggttaagcttggaggagagacactgacggtgtctcaagtggcggggatcgcagctgctaatgacagcaccaccgtgacggtggagctgtcggaggcggcgagggctggagtgaaggcgagcagtgattgggttatggagagcatgaacaaagggactgatagttatggtgttaccaccggcttcggcgccacctctcaccggagaaccaagcaaggcggtgctttacagaaggagctcattagatttttgaacgccggaatattcggtaatggaacggaatctagccacaccctaccacactcagccacaagagccgccatgcttgtcagaatcaacacccttctccagggatactccggcattcgattcgagatcttggaagctatcaccaagttcctcaataacaacatcactccttgtttacccctccgtgggaccatcaccgcctccggtgaccttgttccattatcttacatcgctggtctcctcaccggccgcccaaactcaaaggccgtcggtccaaccggagaaatcctcaatgccgaaaaggcattcgctgctgccggtgtcgaaggtggtttcttcgagttacagcctaaagaagggctagcacttgttaacggcaccgccgtgggatccgggatggcgtcgatggttctcttcgaagctaatgtacttgcgttgttgtcggaagtgttatcggcgatcttcgctgaagttatgcaagggaagccggagttcaccgaccacttaacacacaaattgaagcaccaccccggccaaatcgaagccgccgccatcatggaatacattttggacggaagcgattacgtcaaggcggcgcaaaaggtacacgaaatggaccccttacagaaaccaaaacaagaccgttacgctctccggacatcgccccaatggctcggaccacacattgaagtaatccgatcatcaaccaaaatgatcgagagggaaatcaactccgtcaacgacaatccactcatcgacgtttccagaaacaaagccttacacggtggcaacttccaaggaactccaatcggtgtttccatggacaacacccgtctagccatcgcttccatcggaaaactcatgttcgcccaattttctgaactcgttaacgatttctacaacaatggattaccgtcaaatctctccggcggtcgtaaccctagcttggattacgggttcaaaggtggagaaatcgccatggcttcttattgctcggagctccaatttctcgcgaacccagtcaccaaccacgttcaaagcgccgaacaacacaatcaagacgttaactctttgggcttaatttcagcgagaaaaactcaagaagctgtcgagatcttaaaactcatgtcctccacatatttggtcgctctatgccaatccatcgatttacgccatttggaagaaaacatgaaatcgacagtgaagaacaccgtcagccaagtcgcgaaaaaggtcctaacaatgggcgtcaacggcgagctccacccttccagattctgcgaaaaggatttactccgtgttgttgatcgcgagtacgtcttcgcctacatcgacgacgcttgcagcgccacctacccgttaatgcaaaagctccgtcaagttctcgtcgaccacgccctaaacaacggcgaaacagagaagaacaccagcacctccattttccaaaagatcgccaccttcgaagacgaattaaaagcacttttaccgaaagaagtagaagctgtcagaatcgcgtacgaaaacgacacattaccgatcgcgaacagaatcaaagcctgcagatcgtacccgttgtacaggtttgtcagggaggagctcggcggagtgtttttgaccggcgagaaggtgacgtcgccaggggaggagttcgacaaggtgtttaccgccatgtgcaagggtcaaatcatcgatccgttgttggaatgtgttgaaggctggaatggtgaacctcttccgatttgttag

SEQ ID NO: 2 - protein, 711 aa, Cichorium endivia
MENGNHVNGVVKEFCIKDPLNWGVAAEALTGSHLDEVKKMVKEFRKPVVKLGGETLTVSQVAGIAAANDSTTVTVELSEAARAGVKASSDWVMESMNKGTDSYGVTTGFGATSHRRTKQGGALQKELIRFLNAGIFGNGTESSHTLPHSATRAAMLVRINTLLQGYSGIRFEILEAITKFLNNNITPCLPLRGTITASGDLVPLSYIAGLLTGRPNSKAVGPTGEILNAEKAFAAAGVEGGFFELQPKEGLALVNGTAVGSGMASMVLFEANVLALLSEVLSAIFAEVMQGKPEFTDHLTHKLKHHPGQIEAAAIMEYILDGSDYVKAAQKVHEMDPLQKPKQDRYALRTSPQWLGPHIEVIRSSTKMIEREINSVNDNPLIDVSRNKALHGGNFQGTPIGVSMDNTRLAIASIGKLMFAQFSELVNDFYNNGLPSNLSGGRNPSLDYGFKGGEIAMASYCSELQFLANPVTNHVQSAEQHNQDVNSLGLISARKTQEAVEILKLMSSTYLVALCQSIDLRHLEENMKSTVKNTVSQVAKKVLTMGVNGELHPSRFCEKDLLRVVDREYVFAYIDDACSATYPLMQKLRQVLVDHALNNGETEKNTSTSIFQKIATFEDELKALLPKEVEAVRIAYENDTLPIANRIKACRSYPLYRFVREELGGVFLTGEKVTSPGEEFDKVFTAMCKGQIIDPLLECVEGWNGEPLPIC

SEQ ID NO: 3 - DNA, 2136 bp, Cichorium endivia
atggagaacggtaatcatgttaatggagtcgttaaggagttttgcatcaaggatccgttgaactgaggggttgcggcggaggcgttgaccgggagtcaccttgatgaggtgaagaagatggtgaaggagttcaggaagccggtggttaagcttggaggagagacactgacggtgtctcaagtggcggggatcgcagctgctaatgacagcaccaccgtgacggtggagctgtcggaggcggcgagggctggagtgaaggcgagcagtgattgggttatggagagcatgaacaaagggactgatagttatggtgttaccaccggcttcggcgccacctctcaccggagaaccaagcaaggcggtgctttacagaaggagctcattagatttttgaacgccggaatattcggtaatggaacggaatctagccacaccctaccacactcagccacaagagccgccatgcttgtcagaatcaacacccttctccagggatactccggcattcgattcgagatcttggaagctatcaccaagttcctcaataacaacatcactccttgtttacccctccgtgggaccatcaccgcctccggtgaccttgttccattatcttacatcgctggtctcctcaccggccgcccaaactcaaaggccgtcggtccaaccggagaaatcctcaatgccgaaaaggcattcgctgctgccggtgtcgaaggtggtttcttcgagttacagcctaaagaagggctagcacttgttaacggcaccgccgtgggatccgggatggcgtcgatggttctcttcgaagctaatgtacttgcgttgttgtcggaagtgttatcggcgatcttcgctgaagttatgcaagggaagccggagttcaccgaccacttaacacacaaattgaagcaccaccccggccaaatcgaagccgccgccatcatggaatacattttggacggaagcgattacgtcaaggcggcgcaaaaggtacacgaaatggaccccttacagaaaccaaaacaagaccgttacgctctccggacatcgccccaatggctcggaccacacattgaagtaatccgatcatcaaccaaaatgatcgagagggaaatcaactccgtcaacgacaatccactcatcgacgtttccagaaacaaagccttacacggtggcaacttccaaggaactccaatcggtgtttccatggacaacacccgtctagccatcgcttccatcggaaaactcatgttcgcccaattttctgaactcgttaacgatttctacaacaatggattaccgtcaaatctctccggcggtcgtaaccctagcttggattacgggttcaaaggtggagaaatcgccatggcttcttattgctcggagctccaatttctcgcgaacccagtcaccaaccacgttcaaagcgccgaacaacacaatcaagacgttaactctttgggcttaatttcagcgagaaaaactcaagaagctgtcgagatcttaaaactcatgtcctccacatatttggtcgctctatgccaatccatcgatttacgccatttggaagaaaacatgaaatcgacagtgaagaacaccgtcagccaagtcgcgaaaaaggtcctaacaatgggcgtcaacggcgagctccacccttccagattctgcgaaaaggatttactccgtgttgttgatcgcgagtacgtcttcgcctacatcgacgacgcttgcagcgccacctacccgttaatgcaaaagctccgtcaagttctcgtcgaccacgccctaaacaacggcgaaacagagaagaacaccagcacctccattttccaaaagatcgccaccttcgaagacgaattaaaagcacttttaccgaaagaagtagaagctgtcagaatcgcgtacgaaaacgacacattaccgatcgcgaacagaatcaaagcctgcagatcgtacccgttgtacaggtttgtcagggaggagctcggcggagtgtttttgaccggcgagaaggtgacgtcgccaggggaggagttcgacaaggtgtttaccgccatgtgcaagggtcaaatcatcgatccgttgttggaatgtgttgaaggctggaatggtgaacctcttccgatttgttag

SEQ ID NO: 4 - protein, 21 aa, Cichorium endivia
MENGNHVNGVVKEFCIKDPLN